European Patent Specification EP 3 838 296 B1, published July 16, 2025. Title: VIRAL VECTORS FOR PROPHYLAXIS AND THERAPY OF HEMOGLOBINOPATHIES. Applicant: Cornell University THE CHILDREN'S HOSPITAL OF PHILADELPHIA. The sequence listing filed with the application follows.

SEQUENCE LISTING (29 sequences)

SEQ ID NO: 1 - DNA, 2875 bp, artificial sequence
  ZF-Ldb1 vector as DNA equivalent of RNA lentivirus
cgcgttcgaaggggcaaccaggggtccgcgcgccgaggcctggggagcggggcctcctggggttgggggaggaggtgctcttgtaatctgcggtggtccccaggcgggcgccacccctccgcccgcccgtgccgggagcgcccggcccgacagcaagcgcctctggggccgataaggccctcgggggcctggcccgcacgtcacaggccccgcagaggctgcggtgagtccgccagccccagctgctcctcctcaagcccccaaggcccttcggcggcaattcccaccggtcgccaccatggcccaggcggccttggagcccggagagaaaccctacaaatgcccggagtgtggaaagtccttcagcgactgtagggacctggcacgccaccagcgaacccacacaggcgagaagccctataaatgtccagagtgtggaaagagcttctctagaaacgatgcactgactgagcaccaacgcacccataccggggaaaaaccttataaatgtcctgagtgtggtaaaagtttttctcaattggctcatctccgcgctcaccaacgcacgcatactggtgagaagccctataagtgccccgaatgcggcaagagtttttctcaaagcggggaccttagaagacaccaaagaacccataccggcgaaaaaccttacaagtgtcccgagtgcggaaaatctttttcacgcaaagacaatttgaagaaccaccagcggacacacaccggtgaaaagccttacaaatgtcccgaatgtggcaagtcattctcagaccccggagccctggtgcgccatcagcgcactcacactggcaagaagactagcggccaggccggccaggctagcccgaaaaagaaacgcaaagttgggcgcgccctggatcgggatgtgggcccaactcccatgtacccacctacatacctggagcctgggatcgggaggcacacaccatatggtaaccaaaccgactatagaatatttgagcttaacaaacggctacagaactggacagaggagtgtgacaatctctggtgggatgctttcacaactgagttctttgaagatgacgccatgctgaccatcactttctgcttggaggatggaccaaagagatataccattggccggaccctgataccacgctacttccgaagcatttttgaggggggtgccacagagctgtactacgtgctcaagcaccccaaggaggcattccacagcaacttcgtgtccctcgactgtgaccagggcagcatggtgacccagcacggcaaacccatgtttacccaggtgtgtgtggaaggccggttgtacctggagttcatgtttgacgacatgatgcggataaagacgtggcacttcagcatccggcaacacagagagctcatccccagaagtatcctggccatgcacgcccaggacccccagatgctggatcagctgtccaaaaacattacccggtgtgggctgtccttaattaactacccgtacgacgttccggactacgcttcttgaatcggtaggaattaattctgcagcggccgcggatccgcccctctccctcccccccccctaacgttactggccgaagccgcttggaataaggccggtgtgcgtttgtctatatgttattttccaccatattgccgtcttttggcaatgtgagggcccggaaacctggccctgtcttcttgacgagcattcctaggggtctttcccctctcgccaaaggaatgcaaggtctgttgaatgtcgtgaaggaagcagttcctctggaagcttcttgaagacaaacaacgtctgtagcgaccctttgcaggcagcggaaccccccacctggcgacaggtgcctctgcggccaaaagccacgtgtataagatacacctgcaaaggcggcacaaccccagtgccacgttgtgagttggatagttgtggaaagagtcaaatggctctcctcaagcgtattcaacaaggggctgaaggatgcccagaaggtaccccattgtatgggatctgatctggggcctcggtgcacatgctttacatgtgtttagtcgaggttaaaaaaacgtctaggccccccgaaccacggggacgtggttttcctttgaaaaacacgatgataatatggccacaaccatggtgagcaagggcgaggagctgttcaccggggtggtgcccatcctggtcgagctggacggcgacgtaaacggccacaagttcagcgtgtccggcgagggcgagggcgatgccacctacggcaagctgaccctgaagttcatctgcaccaccggcaagctgcccgtgccctggcccaccctcgtgaccaccctgacctacggcgtgcagtgcttcagccgctaccccgaccacatgaagcagcacgacttcttcaagtccgccatgcccgaaggctacgtccaggagcgcaccatcttcttcaaggacgacggcaactacaagacccgcgccgaggtgaagttcgagggcgacaccctggtgaaccgcatcgagctgaagggcatcgacttcaaggaggacggcaacatcctggggcacaagctggagtacaactacaacagccacaacgtctatatcatggccgacaagcagaagaacggcatcaaggtgaacttcaagatccgccacaacatcgaggacggcagcgtgcagctcgccgaccactaccagcagaacacccccatcggcgacggccccgtgctgctgcccgacaaccactacctgagcacccagtccgccctgagcaaagaccccaacgagaagcgcgatcacatggtcctgctggagttcgtgaccgccgccgggatcactctcggcatggacgagctgtacaagtaa

SEQ ID NO: 2 - protein, 390 aa, artificial sequence
  ZF-LDB1 fusion
MAQAALEPGEKPYKCPECGKSFSDCRDLARHQRTHTGEKPYKCPECGKSFSRNDALTEHQRTHTGEKPYKCPECGKSFSQLAHLRAHQRTHTGEKPYKCPECGKSFSQSGDLRRHQRTHTGEKPYKCPECGKSFSRKDNLSFSDPGALVRHQRTHTGKKTSGQAGQASPKKKRKVGRALDRDVGPTPMYPPTYLEPGIGRHTPYGNQTDYRIFELNKRLQNWTEECDNLWWDAFTTEFFEDDAMLTITFCLEDGPKRYTIGRTLIPRYFRSIFEGGATELYYVLKHPKEAFHSNFVSLDCDQGSMVTQHGKPMFTQVCVEGRLYLEFMFDDMMRIKTWHFSIRQHRELIPRSILAMHAQDPQMLDQLSKNITRCGLSLINYPYDVPDYAS

SEQ ID NO: 3 - DNA, 13550 bp, artificial sequence
  ALS10 as DNA equilvalent of RNA lentiviral vector
ctgtcagaccaagtttactcatatatactttagattgatttaaaacttcatttttaatttaaaaggatctaggtgaagatcctttttgataatctcatgaccaaaatcccttaacgtgagttttcgttccactgagcgtcagaccccgtagaaaagatcaaaggatcttcttgagatcctttttttctgcgcgtaatctgctgcttgcaaacaaaaaaaccaccgctaccagcggtggtttgtttgccggatcaagagctaccaactctttttccgaaggtaactggcttcagcagagcgcagataccaaatactgtccttctagtgtagccgtagttaggccaccacttcaagaactctgtagcaccgcctacatacctcgctctgctaatcctgttaccagtggctgctgccagtggcgataagtcgtgtcttaccgggttggactcaagacgatagttaccggataaggcgcagcggtcgggctgaacggggggttcgtgcacacagcccagcttggagcgaacgacctacaccgaactgagatacctacagcgtgagctatgagaaagcgccacgcttcccgaagggagaaaggcggacaggtatccggtaagcggcagggtcggaacaggagagcgcacgagggagcttccagggggaaacgcctggtatctttatagtcctgtcgggtttcgccacctctgacttgagcgtcgatttttgtgatgctcgtcaggggggcggagcctatggaaaaacgccagcaacgcggcctttttacggttcctggccttttgctggccttttgctcacatgttctttcctgcgttatcccctgattctgtggataaccgtattaccgcctttgagtgagctgataccgctcgccgcagccgaacgaccgagcgcagcgagtcagtgagcgaggaagcggaagagcgcccaatacgcaaaccgcctctccccgcgcgttggccgattcattaatgcagctggcacgacaggtttcccgactggaaagcgggcagtgagcgcaacgcaattaatgtgagttagctcactcattaggcaccccaggctttacactttatgcttccggctcgtatgttgtgtggaattgtgagcggataacaatttcacacaggaaacagctatgaccatgattacgccaagcgcgcaattaaccctcactaaagggaacaaaagctggagctgcaagcttggccattgcatacgttgtatccatatcataatatgtacatttatattggctcatgtccaacattaccgccatgttgacattgattattgactagttattaatagtaatcaattacggggtcattagttcatagcccatatatggagttccgcgttacataacttacggtaaatggcccgcctggctgaccgcccaacgacccccgcccattgacgtcaataatgacgtatgttcccatagtaacgccaatagggactttccattgacgtcaatgggtggagtatttacggtaaactgcccacttggcagtacatcaagtgtatcatatgccaagtacgccccctattgacgtcaatgacggtaaatggcccgcctggcattatgcccagtacatgaccttatgggactttcctacttggcagtacatctacgtattagtcatcgctattaccatggtgatgcggttttggcagtacatcaatgggcgtggatagcggtttgactcacggggatttccaagtctccaccccattgacgtcaatgggagtttgttttggcaccaaaatcaacgggactttccaaaatgtcgtaacaactccgccccattgacgcaaatgggcggtaggcgtgtacggtgggaggtctatataagcagagctcgtttagtgaaccggggtctctctggttagaccagatctgagcctgggagctctctggctaactagggaacccactgcttaagcctcaataaagcttgccttgagtgcttcaagtagtgtgtgcccgtctgttgtgtgactctggtaactagagatccctcagacccttttagtcagtgtggaaaatctctagcagtggcgcccgaacagggacctgaaagcgaaagggaaaccagagctctctcgacgcaggactcggcttgctgaagcgcgcacggcaagaggcgaggggcggcgactggtgagtacgccaaaaattttgactagcggaggctagaaggagagagatgggtgcgagagcgtcagtattaagcgggggagaattagatcgcgatgggaaaaaattcggttaaggccagggggaaagaaaaaatataaattaaaacatatagtatgggcaagcagggagctagaacgattcgcagttaatcctggcctgttagaaacatcagaaggctgtagacaaatactgggacagctacaaccatcccttcagacaggatcagaagaacttagatcattatataatacagtagcaaccctctattgtgtgcatcaaaggatagagataaaagacaccaaggaagctttagacaagatagaggaagagcaaaacaaaagtaagaccaccgcacagcaagcggccgctgatcttcagacctggaggaggagatatgagggacaattggagaagtgaattatataaatataaagtagtaaaaattgaaccattaggagtagcacccaccaaggcaaagagaagagtggtgcagagagaaaaaagagcagtgggaataggagctttgttccttgggttcttgggagcagcaggaagcactatgggcgcagcctcaatgacgctgacggtacaggccagacaattattgtctggtatagtgcagcagcagaacaatttgctgagggctattgaggcgcaacagcatctgttgcaactcacagtctggggcatcaagcagctccaggcaagaatcctggctgtggaaagatacctaaaggatcaacagctcctggggatttggggttgctctggaaaactcatttgcaccactgctgtgccttggaatgctagttggagtaataaatctctggaacagatttggaatcacacgacctggatggagtgggacagagaaattaacaattacacaagcttaatacactccttaattgaagaatcgcaaaaccagcaagaaaagaatgaacaagaattattggaattagataaatgggcaagtttgtggaattggtttaacataacaaattggctgtggtatataaaattattcataatgatagtaggaggcttggtaggtttaagaatagtttttgctgtactttctatagtgaatagagttaggcagggatattcaccattatcgtttcagacccacctcccaaccccgaggggacccgacaggcccgaaggaatagaagaagaaggtggagagagagacagagacagatccattcgattagtgaacggatctcgacggtatcggttaacttttaaaagaaaaggggggattggggggtacagtgcaggggaaagaatagtagacataatagcaacagacatacaaactaaagaattacaaaaacaaattacaaaaattcaaaattttatcgataagcttgggagttccgcgtgttgggggtggaccatcctctaggtattgaataagaaaaatgaagttaaggtggttgatggtaacactatgctaataactgcagagccagaagcaccataagggacatgataagggagccagcagacctctgatctcttcctgaatgctaatcttaaacatcctgaggaagaatgggacttccatttggggtgggcctatgatagggtaataagacagtagtgaatatcaagctacaaaaagccccctttcaaattcttctcagtcctaacttttcatactaagcccagtccttccaaagcagactgtgaaagagtgatagttccgggagactagcactgcagattccgggtcactgtgagtgggggaggcagggaagaagggctcacaggacagtcaaaccatgccccctgtttttccttcttcaagtagacctctataagacaacagagacaactaaggctgagtggccaggcgaggagaaaccatctcgccgtaaaacatggaaggaacacttcaggggaaaggtggtatctctaagcaagagaactgagtggagtcaaggctgagagatgcaggataagcaaatgggtagtgaaaagacattcatgaggacagctaaaacaataagtaatgtaaaatacagcatagcaaaactttaacctccaaatcaagcctctacttgaatccttttctgagggatgaataaggcataggcatcaggggctgttgccaatgtgcattagctgtttgcagcctcaccttctttcatggagtttaagatatagtgtattttcccaaggtttgaactagctcttcatttctttatgttttaaatgcactgacctcccacattccctttttagtaaaatattcagaaataatttaaatacatcattgcaatgaaaataaatgttttttattaggcagaatccagatgctcaaggcccttcataatatcccccagtttagtagttggacttagggaacaaaggaacctttaatagaaattggacagcaagaaagcgagcttagtgatacttgtgggccagggcattagccacaccagccaccactttctgataggcagcctgcactggtggggtgaattctttgccaaagtgatgggccagcacacagaccagcacgttgcccaggagctgtgggaggaagataagaggtatgaacatgattagcaaaagggcctagcttggactcagaataatccagccttatcccaaccataaaataaaagcagaatggtagctggattgtagctgctattagcaatatgaaacctcttacatcagttacaatttatatgcagaaatatttatatgcagaaatattgctattgccttaacccagaaattatcactgttattctttagaatggtgcaaagaggcatgatacattgtatcattattgccctgaaagaaagagattagggaaagtattagaaataagataaacaaaaaagtatattaaaagaagaaagcattttttaaaattacaaatgcaaaattaccctgatttggtcaatatgtgtacacatattaaaacattacactttaacccataaatatgtataatgattatgtatcaattaaaaataaaagaaaataaagtagggagattatgaatatgcaaataagcacacatatattccaaatagtaatgtactaggcagactgtgtaaagtttttttttaagttacttaatgtatctcagagatatttccttttgttatacacaatgttaaggcattaagtataatagtaaaaattgcggagaagaaaaaaaaagaaagcaagaattaaacaaaagaaaacaattgttatgaacagcaaataaaagaaactaaaacgatcctgagacttccacactgatgcaatcattcgtctgtttcccattctaaactgtaccctgttacttctccccttcctatgacatgaacttaaccatagaaaagaaggggaaagaaaacatcaagggtcccatagactcaccctgaagttctcaggatccacgtgcagcttgtcacagtgcagctcactcagtgtggcaaaggtgcccttgaggttgtccaggtgagccaggccatcactaaaggcaccgagcactttcttgccatgagccttcaccttagggttgcccataacagcatcaggagtggacagatccccaaaggactcaaagaacctctgggtccaagggtagaccaccagcagcctaagggtgggaaaatagaccaataggcagagagagtcagtgcctatcagaaacccaagagtcttctctgtctccacatgcccagtttctattggtctccttaaacctgtcttgtaaccttgataccaacctgcccagggcctcaccaccaacttcatccacgttcaccttgccccacagggcagtaacggcagacttctcctcaggagtcaggtgcaccatggtgtctgtttgaggttgctagtgaacacagttgtgtcagaagcaaatgtaagcaatagatggctctgccctgacttttatgcccagccctggctcctgccctccctgctcctgggagtagattggccaaccctagggtgtggctccacagggtgaggtctaagtgatgacagccgtacctgtccttggctcttctggcactggcttaggagttggacttcaaaccctcagccctccctctaagatatatctcttggccccataccatcagtacaaattgctactaaaaacatcctcctttgcaagtgtatttacgtaatatttggaatcacagcttggtaagcatattgaagatcgttttcccaattttcttattacacaaataagaaattgatgcactaaaagtggaagagttttgtctaccataattcagctttgggatatgtagatggatctcttcctgcgtctccagaatatgcaaaatacttacaggacagaatggatgaaaactctacctcagttctaagcatatcttctccttatttggattaaaaccttctggtaagaaaagaaaaaaaatatatatatatatgtgtatatatacacacatacatatacatatatatgcattcatttgttgttgtttttcttaatttgctcatggtatatgtgtatatatatatatatatattcaggaaataatatattctagaatatgtcacattctgtctcaggcatccattttctttatgatgccgtttgaggtggagttttagtcaggtggtcagcttctccttttttttgccatctgccctgtaagcatcctgctggggacccagataggagtcatcactctaggctgagaacatctgggcacacaccctaagcctcagcatgactcatcatgactcagcattgctgtgcttgagccagaaggtttgcttagaaggttacacagaaccagaaggcgggggtggggcactgaccccgacaggggcctggccagaactgctcatgcttggactatgggaggtcactaatggagacacacagaaatgtaacaggaactaaggaaaaactgaagcttatttaatcagagatgagatgctggaagggatagagggagctgagcttgtaaaaagtatagtaatcattcagcaaatggttttgaagcacctgctggatgctaaacactattttcagtgcttgaatcataaataagaataaaacatgtatcttattccccacaagagtccaagtaaaaaataacagttaattataatgtgctctgtcccccaggctggagtgcagtggcacgatctcagctcactgcaacctccgcctcccgggttcaagcaattctcctgcctcagccaccctaatagctgggattacaggtgcacaccaccatgccaggctaatttttgtactttttgtagaggcagggtatcaccatgttgtccaagatggtcttgaactcctgagctccaagcagtccacccacctcagcctcccaaagtgctatctgcggccgcctatctgtaccactagtctcgagaagctttcattaaaaaaagtctaaccagctgcattcgactttgactgcagcagctggttagaaggttctactggaggagggtcccagcccattgctaaattaacatcaggctctgagactggcagtatatctctaacagtggttgatgctatcttctggaacttgcctgctacattgagaccactgacccatacataggaagcccatagctctgtcctgaactgttaggccactggtccagagagtgtgcatctcctttgatcctcataataaccctatgagatagacacaattattactcttactttatagatgatgatcctgaaaacataggagtcaaggcacttgcccctagctgggggtataggggagcagtcccatgtagtagtagaatgaaaaatgctgctatgctgtgcctcccccacctttcccatgtctgccctctactcatggtctatctctcctggctcctgggagtcatggactccacccagcaccaccaacctgacctaaccacctatctgagcctgccagcctataacccatctgggccctgatagctggtggccagccctgaccccaccccaccctccctggaacctctgatagacacatctggcacaccagctcgcaaagtcaccgtgagggtcttgtgtttgctgagtcaaaattccttgaaatccaagtccttagagactcctgctcccaaatttacagtcatagacttcttcatggctgtctcctttatccacagaatgattcctttgcttcattgccccatccatctgatcctcctcatcagtgcagcacagggcccatgagcagtagctgcagagtctcacataggtctggcactgcctctgacatgtccgaccttaggcaaatgcttgactcttctgagctcagtcttgtcatggcaaaataaagataataatagtgtttttttatggagttagcgtgaggatggaaaacaatagcaaaattgattagactataaaaggtctcaacaaatagtagtagattttatcatccattaatccttccctctcctctcttactcatcccatcacgtatgcctcttaattttcccttacctataataagagttattcctcttattatattcttcttatagtgattctggatattaaagtgggaatgaggggcaggccactaacgaagaagatgtttctcaaagaagccattctccccacatagatcatctcagcagggttcaggaagataaaggaggatcaaggtcgaaggtaggaactaaggaagaacactgggcaagtggatcctgagccccttttcctctaactgaaagaaggaaaaaaaaaatggaacccaaaatattctacatagtttccatgtcacagccagggctgggcagtctcctgttatttcttttaaaataaatatatcatttaaatgcataaataagcaaaccctgctcgggaatgggagggagagtctctggagtccaccccttctcggccctggctctgcagatagtgctatcaaagccctgacagagccctgcccattgctgggccttggagtgagtcagcctagtagagaggcagggcaagccatctcatagctgctgagtgggagagagaaaagggctcattgtctataaactcaggtcatggctattcttattctcacactaagaaaaagaatgagatgtctacatataccctgcgtcccctcttgtgtactggggcccccaagagctctctaaaagtgatggcaaagtcattgcgctagatgccatcccatctattataaacctgcatttgtctccacacaccagtcatggacaataaccctcctcccaggtccacgtgcttgtctttgtataatactcaagtaatttcggaaaatgtattctttcaatcttgttctgttattcctgtttcaatggcttagtagaaaaagtacatacttgttttcccataaattgacaatagacaatttcacatcaatgtctatatgggtcgttgtgtttgctgtgtttgcaaaaactcacaataactttatattgttactactctaagaaagttacaacatggtgaatacaagagaaagctattacaagtccagaaaataaaagttatcatcttgaggcctcagctttctaggaataatatcaatattacaaaattaatctaacaattatgaacagcaatgagataatatgtacaaagtacccagacctatgtggtagagcatcaaggaagcgcattgcggagcagttttttgtttgtttgtttttgtattctgtttcgtgaggcaaggtttcactctgctgtccaggctggagtgcagtggcaagatcatgtctcactgcagccttgacactacacgtgctttaagaccaatgacttacaaggcagctgtagatcttagccactttttaaaagaaaaggggggactggaagggctaattcactcccaacgaagacaagatctgctttttgctagcgcggccgctctagactagtggggcccgtgcaattgaagccggctggcgccaagcttctctgcaggatgtgcgggccaggcccccgagggccttatcggccccagaggcgcttgctgtcgggccgggcgctcccggcacgggcgggcggaggggtggcgcccgcctggggaccgcagattacaagagcacctcctcccccaaccccaggaggccccgctccccaggcctcggccggcgcggacccctggttgccccggatgtacaggcatgcgtcgacctcgagggggggcccggtaccgctagcactgggtctctctggttagaccagatctgagcctgggagctctctggctaactagggaacccactgcttaagcctcaataaagcttgccttgagtgcttcaagtagtgtgtgcccgtctgttgtgtgactctggtaactagagatccctcagacccttttagtcagtgtggaaaatctctagcaggtcgacaatcaacctctggattacaaaatttgtgaaagattgactggtattcttaactatgttgctccttttacgctatgtggatacgctgctttaatgcctttgtatcatgctattgcttcccgtatggctttcattttctcctccttgtataaatcctggttgctgtctctttatgaggagttgtggcccgttgtcaggcaacgtggcgtggtgtgcactgtgtttgctgacgcaacccccactggttggggcattgccaccacctgtcagctcctttccgggactttcgctttccccctccctattgccacggcggaactcatcgccgcctgccttgcccgctgctggacaggggctcggctgttgggcactgacaattccgtggtgttgtcggggaagctgacgtcctttccatggctgctcgcctgtgttgccacctggattctgcgcgggacgtccttctgctacgtcccttcggccctcaatccagcggaccttccttcccgcggcctgctgccggctctgcggcctcttccgcgtcttcgccttcgccctcagacgagtcggatctccctttgggccgcctccccgcctggaattcgagctcggtacctgatcagcctcgactgtgccttctagttgccagccatctgttgtttgcccctcccccgtgccttccttgaccctggaaggtgccactcccactgtcctttcctaataaaatgaggaaattgcatcgcattgtctgagtaggtgtcattctattctggggggtggggtggggcaggacagcaagggggaggattgggaagacaatagcaggcatgctggggatgcggtgggctctatggcttctgaggaaagaaccagctggggctcgagatccactagttctagcctcgaggctagagcggccgccaccgcggtagtagttcatgtcatcttattattcagtatttataacttgcaaagaaatgaatatcagagagtgagaggaacttgtttattgcagcttataatggttacaaataaagcaatagcatcacaaatttcacaaataaagcatttttttcactgcattctagttgtggtttgtccaaactcatcaatgtatcttatcatgtctggctctagctatcccgcccctaactccgcccagttccgcccattctccgccccatggctgactaattttttttatttatgcagaggccgaggccgcctcggcctctgagctattccagaagtagtgaggaggcttttttggaggcctaggcttttgcgtcgagacgtacccaattcgccctatagtgagtcgtattacgcgcgctcactggccgtcgttttacaacgtcgtgactgggaaaaccctggcgttacccaacttaatcgccttgcagcacatccccctttcgccagctggcgtaatagcgaagaggcccgcaccgatcgcccttcccaacagttgcgcagcctgaatggcgaatggcgcgacgcgccctgtagcggcgcattaagcgcggcgggtgtggtggttacgcgcagcgtgaccgctacacttgccagcgccctagcgcccgctcctttcgctttcttcccttcctttctcgccacgttcgccggctttccccgtcaagctctaaatcgggggctccctttagggttccgatttagtgctttacggcacctcgaccccaaaaaacttgattagggtgatggttcacgtagtgggccatcgccctgatagacggtttttcgccctttgacgttggagtccacgttctttaatagtggactcttgttccaaactggaacaacactcaaccctatctcggtctattcttttgatttataagggattttgccgatttcggcctattggttaaaaaatgagctgatttaacaaaaatttaacgcgaattttaacaaaatattaacgtttacaatttcccaggtggcacttttcggggaaatgtgcgcggaacccctatttgtttatttttctaaatacattcaaatatgtatccgctcatgagacaataaccctgataaatgcttcaataatattgaaaaaggaagagtatgagtattcaacatttccgtgtcgcccttattcccttttttgcggcattttgccttcctgtttttgctcacccagaaacgctggtgaaagtaaaagatgctgaagatcagttgggtgcacgagtgggttacatcgaactggatctcaacagcggtaagatccttgagagttttcgccccgaagaacgttttccaatgatgagcacttttaaagttctgctatgtggcgcggtattatcccgtattgacgccgggcaagagcaactcggtcgccgcatacactattctcagaatgacttggttgagtactcaccagtcacagaaaagcatcttacggatggcatgacagtaagagaattatgcagtgctgccataaccatgagtgataacactgcggccaacttacttctgacaacgatcggaggaccgaaggagctaaccgcttttttgcacaacatgggggatcatgtaactcgccttgatcgttgggaaccggagctgaatgaagccataccaaacgacgagcgtgacaccacgatgcctgtagcaatggcaacaacgttgcgcaaactattaactggcgaactacttactctagcttcccggcaacaattaatagactggatggaggcggataaagttgcaggaccacttctgcgctcggcccttccggctggctggtttattgctgataaatctggagccggtgagcgtgggtctcgcggtatcattgcagcactggggccagatggtaagccctcccgtatcgtagttatctacacgacggggagtcaggcaactatggatgaacgaaatagacagatcgctgagataggtgcctcactgattaagcattggtaa

SEQ ID NO: 4 - DNA, 13550 bp, human; identical to SEQ ID NO: 3

SEQ ID NO: 5 - protein, 147 aa, human
MVHLTPEEKSAVTALWGKVNVDEVGGEALGRLLVVYPWTQRFFESFGDLSTPDAVMGNPKVKAHGKKVLGAFSDGLAHLDNLKGTFATLSELHCDKLHVDPENFRLLGNVLVCVLAHHFGKEFTPPVQAAYQKVVAGVANALAHKYH

SEQ ID NO: 6 - DNA, 20 bp, artificial sequence
  Primer
caagaaagtgctcggtgcct

SEQ ID NO: 7 - DNA, 19 bp, artificial sequence
  Primer
gcaaaggtgcccttgaggt

SEQ ID NO: 8 - DNA, 25 bp, artificial sequence
  Primer
tagtgatggcctggctcacctggac

SEQ ID NO: 9 - DNA, 20 bp, artificial sequence
  Primer
tccccaccaccaagacctac

SEQ ID NO: 10 - DNA, 19 bp, artificial sequence
  Primer
ccttaacctgggcagagcc

SEQ ID NO: 11 - DNA, 22 bp, artificial sequence
  Primer
tcccgcacttcgacctgagcca

SEQ ID NO: 12 - DNA, 21 bp, artificial sequence
  Primer
tggcaagaaggtgctgacttc

SEQ ID NO: 13 - DNA, 19 bp, artificial sequence
  Primer
tcactcagctgggcaaagg

SEQ ID NO: 14 - DNA, 24 bp, artificial sequence
  Primer
tgggagatgccataaagcacctgg

SEQ ID NO: 15 - DNA, 24 bp, artificial sequence
  Primer
tgcgaacttgaacgtcaggagtct

SEQ ID NO: 16 - DNA, 24 bp, artificial sequence
  Primer
tgcgaacttgaacgtcaggagtct

SEQ ID NO: 17 - DNA, 24 bp, artificial sequence
  Primer
agctgctttcggctttctccctta

SEQ ID NO: 18 - DNA, 24 bp, artificial sequence
  Primer
cctttgcatttgcagcagttcagc

SEQ ID NO: 19 - DNA, 24 bp, artificial sequence
  Primer
tcaaccgatcatccctcacactct

SEQ ID NO: 20 - DNA, 24 bp, artificial sequence
  Primer
aatcagcagcgcttccattcaagg

SEQ ID NO: 21 - DNA, 18 bp, artificial sequence
  Primer
gctgcctccacccaagtg

SEQ ID NO: 22 - DNA, 21 bp, artificial sequence
  Primer
accaactctgggcagtcacat

SEQ ID NO: 23 - DNA, 20 bp, artificial sequence
  Primer
agcaaccacccatgcctgcc

SEQ ID NO: 24 - DNA, 20 bp, artificial sequence
  Primer
ctcgggccaaaggcctcacg

SEQ ID NO: 25 - DNA, 17 bp, artificial sequence
  Primer
cggctgttgggcactga

SEQ ID NO: 26 - DNA, 19 bp, artificial sequence
  Primer
ggaaggtccgctggattga

SEQ ID NO: 27 - DNA, 22 bp, artificial sequence
  Primer
atggctgctcgcctgtgttgcc

SEQ ID NO: 28 - DNA, 22 bp, artificial sequence
  Primer
aaggtgagcaaggtggagattc

SEQ ID NO: 29 - DNA, 21 bp, artificial sequence
  Primer
ttccgagttcagctccaactg